European Patent Application EP 4 174 179 A2, published May 3, 2023. Title: RNA Containing Modified Nucleosides and Methods of Use Thereof. Applicant: The Trustees of the University of Pennsylvania. Application EP - not yet assigned. The sequence listing filed with the application follows.

SEQUENCE LISTING (11 sequences)

SEQ ID NO: 1 - RNA, 1864 nt, Photinus pyralis
ggaauucucaacacaacauauacaaaacaaacgaaucucaagcaaucaagcauucuacuucuauugcagcaauuuaaaucauuucuuuuaaagcaaaagcaauuuucugaaaauuuucaccauuuacgaacgauagccauggaagacgccaaaaacauaaagaaaggcccggcgccauucuauccucuagaggauggaaccgcuggagagcaacugcauaaggcuaugaagagauacgcccugguuccuggaacaauugcuuuuacagaugcacauaucgaggugaacaucacguacgcggaauacuucgaaauguccguucgguuggcagaagcuaugaaacgauaugggcugaauacaaaucacagaaucgucguaugcagugaaaacucucuucaauucuuuaugccgguguugggcgcguuauuuaucggaguugcaguugcgcccgcgaacgacauuuauaaugaacgugaauugcucaacaguaugaacauuucgcagccuaccguaguguuuguuuccaaaaagggguugcaaaaaauuuugaacgugcaaaaaaaauuaccaauaauccagaaaauuauuaucauggauucuaaaacggauuaccagggauuucagucgauguacacguucgucacaucucaucuaccucccgguuuuaaugaauacgauuuuguaccagaguccuuugaucgugacaaaacaauugcacugauaaugaauuccucuggaucuacuggguuaccuaaggguguggcccuuccgcauagaacugccugcgucagauucucgcaugccagagauccuauuuuuggcaaucaaaucauuccggauacugcgauuuuaaguguuguuccauuccaucacgguuuuggaauguuuacuacacucggauauuugauauguggauuucgagucgucuuaauguauagauuugaagaagagcuguuuuuacgaucccuucaggauuacaaaauucaaagugcguugcuaguaccaacccuauuuucauucuucgccaaaagcacucugauugacaaauacgauuuaucuaauuuacacgaaauugcuucugggggcgcaccucuuucgaaagaagucggggaagcgguugcaaaacgcuuccaucuuccagggauacgacaaggauaugggcucacugagacuacaucagcuauucugauuacacccgagggggaugauaaaccgggcgcggucgguaaaguuguuccauuuuuugaagcgaagguuguggaucuggauaccgggaaaacgcugggcguuaaucagagaggcgaauuaugugucagaggaccuaugauuauguccgguuauguaaacaauccggaagcgaccaacgccuugauugacaaggauggauggcuacauucuggagacauagcuuacugggacgaagacgaacacuucuucauaguugaccgcuugaagucuuuaauuaaauacaaaggauaucagguggcccccgcugaauuggaaucgauauuguuacaacaccccaacaucuucgacgcgggcguggcaggucuucccgacgaugacgccggugaacuucccgccgccguuguuguuuuggagcacggaaagacgaugacggaaaaagagaucguggauuacguggccagucaaguaacaaccgcgaaaaaguugcgcggaggaguuguguuuguggacgaaguaccgaaaggucuuaccggaaaacucgacgcaagaaaaaucagagagauccucauaaaggccaagaagggcggaaaguccaaauuguaaaauguaacucuagaggauccccaaaaaaaaaaaaaaaaaaaaaaaaaaaaaaaaaaaaaaaaaaaaaaaaaca

SEQ ID NO: 2 - RNA, 1571 nt, Renilla reniformis
ggcuagccaccaugacuucgaaaguuuaugauccagaacaaaggaaacggaugauaacugguccgcaguggugggccagauguaaacaaaugaauguucuugauucauuuauuaauuauuaugauucagaaaaacaugcagaaaaugcuguuauuuuuuuacaugguaacgcggccucuucuuauuuauggcgacauguugugccacauauugagccaguagcgcgguguauuauaccagaccuuauugguaugggcaaaucaggcaaaucugguaaugguucuuauagguuacuugaucauuacaaauaucuuacugcaugguuugaacuucuuaauuuaccaaagaagaucauuuuugucggccaugauuggggugcuuguuuggcauuucauuauagcuaugagcaucaagauaagaucaaagcaauaguucacgcugaaaguguaguagaugugauugaaucaugggaugaauggccugauauugaagaagauauugcguugaucaaaucugaagaaggagaaaaaaugguuuuggagaauaacuucuucguggaaaccauguugccaucaaaaaucaugagaaaguuagaaccagaagaauuugcagcauaucuugaaccauucaaagagaaaggugaaguucgucguccaacauuaucauggccucgugaaaucccguuaguaaaaggugguaaaccugacguuguacaaauuguuaggaauuauaaugcuuaucuacgugcaagugaugauuuaccaaaaauguuuauugaaucggacccaggauucuuuuccaaugcuauuguugaaggugccaagaaguuuccuaauacugaauuugucaaaguaaaaggucuucauuuuucgcaagaagaugcaccugaugaaaugggaaaauauaucaaaucguucguugagcgaguucucaaaaaugaacaaaugucgacgggggccccuaggaauuuuuuagggaagaucuggccuuccuacaagggaaggccagggaauuuucuucagagcagaccagagccaacagccccaccagaagagagcuucaggucugggguagagacaacaacucccccucagaagcaggagccgauagacaaggaacuguauccuuuaacuucccucagaucacucuuuggcaacgaccccucgucacaauaaagauaggggggcaacuaaagggaucggccgcuucgagcagacaugauaagauacauugaugaguuuggacaaaccacaacuagaaugcagugaaaaaaaugcuuuauuugugaaauuugugaugcuauugcuuuauuuguaaccauuauaagcugcaauaaacaaguuaacaacaacaauugcauucauuuuauguuucagguucagggggaggugugggagguuuuuuaaagcaaguaaaaccucuacaaaugugguaaaaucgauaaguuuaaacagauccagguggcacuuuucggggaaaugugcgcggaaccccuauuuguuuauuuuucuaaauacauucaaauauguauccgcucaugagacaauaacccugauaaaugcuucaauaau

SEQ ID NO: 3 - RNA, 726 nt, Homo sapiens
gggaauuuggcccucgaggccaagaauucggcacgaggcacgcggccagccagcagacagaggacucucauuaaggaagguguccugugcccugacccuacaagaugccaagagaagaugcucacuucaucuaugguuaccccaagaaggggcacggccacucuuacaccacggcugaagaggccgcugggaucggcauccugacagugauccugggagucuuacugcucaucggcuguugguauuguagaagacgaaauggauacagagccuugauggauaaaagucuucauguuggcacucaaugugccuuaacaagaagaugcccacaagaaggguuugaucaucgggacagcaaagugucucuucaagagaaaaacugugaaccugugguucccaaugcuccaccugcuuaugagaaacucucugcagaacagucaccaccaccuuauucaccuuaagagccagcgagacaccugagacaugcugaaauuauuucucucacacuuuugcuugaauuuaauacagacaucuaauguucuccuuuggaaugguguaggaaaaaugcaagccaucucuaauaauaagucaguguuaaaauuuuaguagguccgcuagcaguacuaaucaugugaggaaaugaugagaaauauuaaauugggaaaacuccaucaauaaauguugcaaugcaugauaaaaaaaaaaaaaaaaaaaacugcggccgca

SEQ ID NO: 4 - RNA, 712 nt, Homo sapiens
gggaauaagcuugcggccgcaguuuuuuuuuuuuuuuuuuuuaucaugcauugcaacauuuauugauggaguuuucccaauuuaauauuucucaucauuuccucacaugauuaguacugcuagcggaccuacuaaaauuuuaacacugacuuauuauuagagauggcuugcauuuuuccuacaccauuccaaaggagaacauuagaugucuguauaaauucaagcaaaagugugagagaaauaauuucagcaugucucaggugucucgcuggcucuuaaggugaauaaggugguggugacuguucugcagagaguuucucauaagcagguggagcauugggaaccacagguucacaguuuuucucuugaagagacacuuugcugucccgaugaucaaacccuucuugugggcaucuucuuguuaaggcacauugagugccaacaugaagacuuuuauccaucaaggcucuguauccauuucgucuucuacaauaccaacagccgaugagcaguaagacucccaggaucacugucaggaugccgaucccagcggccucuucagccgugguguaagaguggccgugccccuucuugggguaaccauagaugaagugagcaucuucucuuggcaucuuguagggucagggcacaggacaccuuccuuaaugagaguccucugucugcuggcuggccgcgugccucgugccgaauu

SEQ ID NO: 5 - RNA, 494 nt, Homo sapiens
gggagacccaagcuggcuagcagucauccaacagaaucaugagacagacuuugccuuguaucuacuuuugggggggccuuuugcccuuugggaugcugugugcauccuccaccaccaagugcacuguuagccaugaaguugcugacugcagccaccugaaguugacucagguacccgaugaucuacccacaaacauaacaguguugaaccuuacccauaaucaacucagaagauuaccagccgccaacuucacaagguauagccagcuaacuagcuuggauguaggauuuaacaccaucucaaaacuggagccagaauugugccagaaacuucccauguuaaaaguuuugaaccuccagcacaaugagcuaucucaacuuucugauaaaaccuuugccuucugcacgaauuugacugaacuccaucucauguccaacucaauccagaaaauuaaaaauaaucccuuugucaagcagaagaauuuaaucacauua

SEQ ID NO: 6 - RNA, 21 nt, Artificial Sequence
  Chemically synthesized
uggauccggcuuugagaucuu

SEQ ID NO: 7 - RNA, 21 nt, Artificial Sequence
  Chemically synthesized
  modified_base (11)..(11): um
uggauccggcuuugagaucuu

SEQ ID NO: 8 - RNA, 21 nt, Artificial Sequence
  Chemically synthesized
  modified_base (6)..(6): m5c
uggauccggcuuugagaucuu

SEQ ID NO: 9 - RNA, 21 nt, Artificial Sequence
  Chemically synthesized
  modified_base (12)..(12): p
uggauccggcuuugagaucuu

SEQ ID NO: 10 - RNA, 31 nt, Artificial Sequence
  Chemically synthesized
gggagacagggguguccgccauuuccagguu

SEQ ID NO: 11 - RNA, 31 nt, Artificial Sequence
  Chemically synthesized
gggagacaggcuauaacucacauaauguauu